European Patent Application EP 4 316 519 A2, published February 7, 2024. Title: ANTIBODIES WITH MODULATED GLYCAN PROFILES. Applicant: AMGEN INC. Application EP. The sequence listing filed with the application follows.

SEQUENCE LISTING (6 sequences)

SEQ ID NO: 1 - protein, 448 aa, Homo sapiens
EVQLLESGGGLVQPGGSLRLSCAASGFTFSSYAMSWVRQAPGKGLEWVSGITGSGGSTYYADSVKGRFTISRDNSKNTLYLQMNSLRAEDTAVYYCAKDPGTTVIMSWFDPWGQGTLVTVSSASTKGPSVFPLAPCSRSTSESTAALGCLVKDYFPEPVTVSWNSGALTSGVHTFPAVLQSSGLYSLSSVVTVPSSNFGTQTYTCNVDHKPSNTKVDKTVERKCCVECPPCPAPPVAGPSVFLFPPKPKDTLMISRTPEVTCVVVDVSHEDPEVQFNWYVDGVEVHNAKTKPREEQFNSTFRVVSVLTVVHQDWLNGKEYKCKVSNKGLPAPIEKTISKTKGQPREPQVYTLPPSREEMTKNQVSLTCLVKGFYPSDIAVEWESNGQPENNYKTTPPMLDSDGSFFLYSKLTVDKSRWQQGNVFSCSVMHEALHNHYTQKSLSLSPGK

SEQ ID NO: 2 - protein, 215 aa, Homo sapiens
EIVLTQSPGTLSLSPGERATLSCRASQSVRGRYLAWYQQKPGQAPRLLIYGASSRATGIPDRFSGSGSGTDFTLTISRLEPEDFAVFYCQQYGSSPRTFGQGTKVEIKRTVAAPSVFIFPPSDEQLKSGTASVVCLLNNFYPREAKVQWKVDNALQSGNSQESVTEQDSKDSTYSLSSTLTLSKADYEKHKVYACEVTHQGLSSPVTKSFNRGEC

SEQ ID NO: 3 - DNA, 1401 bp, Homo sapiens
  source 1..1401: mol_type = other DNA
atggagtttgggctgagctggctttttcttgtggctattttaaaaggtgtccagtgtgaggtgcagctgttggagtctgggggaggcttggtacagcctggggggtccctgagactctcctgtgcagcctctggattcacctttagcagctatgccatgagctgggtccgccaggctccagggaaggggctggagtgggtctcaggtattactgggagtggtggtagtacatactacgcagactccgtgaagggccggttcaccatctccagagacaattccaagaacacgctgtatctgcaaatgaacagcctgagagccgaggacacggccgtatattactgtgcgaaagatccagggactacggtgattatgagttggttcgacccctggggccagggaaccctggtcaccgtctcctcagcctccaccaagggcccatcggtcttccccctggcgccctgctccaggagcacctccgagagcacagcggccctgggctgcctggtcaaggactacttccccgaaccggtgacggtgtcgtggaactcaggcgctctgaccagcggcgtgcacaccttcccagctgtcctacagtcctcaggactctactccctcagcagcgtggtgaccgtgccctccagcaacttcggcacccagacctacacctgcaacgtagatcacaagcccagcaacaccaaggtggacaagacagttgagcgcaaatgttgtgtcgagtgcccaccgtgcccagcaccacctgtggcaggaccgtcagtcttcctcttccccccaaaacccaaggacaccctcatgatctcccggacccctgaggtcacgtgcgtggtggtggacgtgagccacgaagaccccgaggtccagttcaactggtacgtggacggcgtggaggtgcataatgccaagacaaagccacgggaggagcagttcaacagcacgttccgtgtggtcagcgtcctcaccgttgtgcaccaggactggctgaacggcaaggagtacaagtgcaaggtctccaacaaaggcctcccagcccccatcgagaaaaccatctccaaaaccaaagggcagccccgagaaccacaggtgtacaccctgcccccatcccgggaggagatgaccaagaaccaggtcagcctgacctgcctggtcaaaggcttctaccccagcgacatcgccgtggagtgggagagcaatgggcagccggagaacaactacaagaccacacctcccatgctggactccgacggctccttcttcctctacagcaagctcaccgtggacaagagcaggtggcagcaggggaacgtcttctcatgctccgtgatgcatgaggctctgcacaaccactacacgcagaagagcctctccctgtctccgggtaaa

SEQ ID NO: 4 - DNA, 705 bp, Homo sapiens
  source 1..705: mol_type = other DNA
atggaaaccccagcgcagcttctcttcctcctgctactctggctcccagataccaccggagaaattgtgttgacgcagtctccaggcaccctgtctttgtctccaggggaaagagccaccctctcctgtagggccagtcagagtgttcgcggcaggtacttagcctggtaccagcagaaacctggccaggctcccaggctcctcatctatggtgcatccagcagggccactggcatcccagacaggttcagtggcagtgggtctgggacagacttcactctcaccatcagcagactggagcctgaagattttgcagtgttttactgtcagcagtatggtagttcacctcggacgttcggccaagggaccaaggtggaaatcaaacgaactgtggctgcaccatctgtcttcatcttcccgccatctgatgagcagttgaaatctggaactgcctctgttgtgtgcctgctgaataacttctatcccagagaggccaaagtacagtggaaggtggataacgccctccaatcgggtaactcccaggagagtgtcacagagcaggacagcaaggacagcacctacagcctcagcagcaccctgacgctgagcaaagcagactacgagaaacacaaagtctacgcctgcgaagtcacccatcagggcctgagctcgcccgtcacaaagagcttcaacaggggagagtgt

SEQ ID NO: 5 - protein, 467 aa, Homo sapiens
MEFGLSWLFLVAILKGVQCEVQLLESGGGLVQPGGSLRLSCAASGFTFSSYAMSWVRQAPGKGLEWVSGITGSGGSTYYADSVKGRFTISRDNSKNTLYLQMNSLRAEDTAVYYCAKDPGTTVIMSWFDPWGQGTLVTVSSASTKGPSVFPLAPCSRSTSESTAALGCLVKDYFPEPVTVSWNSGALTSGVHTFPAVLQSSGLYSLSSVVTVPSSNFGTQTYTCNVDHKPSNTKVDKTVERKCCVECPPCPAPPVAGPSVFLFPPKPKDTLMISRTPEVTCVVVDVSHEDPEVQFNWYVDGVEVHNAKTKPREEQFNSTFRVVSVLTVVHQDWLNGKEYKCKVSNKGLPAPIEKTISKTKGQPREPQVYTLPPSREEMTKNQVSLTCLVKGFYPSDIAVEWESNGQPENNYKTTPPMLDSDGSFFLYSKLTVDKSRWQQGNVFSCSVMHEALHNHYTQKSLSLSPGK

SEQ ID NO: 6 - protein, 235 aa, Homo sapiens
METPAQLLFLLLLWLPDTTGEIVLTQSPGTLSLSPGERATLSCRASQSVRGRYLAWYQQKPGQAPRLLIYGASSRATGIPDRFSGSGSGTDFTLTISRLEPEDFAVFYCQQYGSSPRTFGQGTKVEIKRTVAAPSVFIFPPSDEQLKSGTASVVCLLNNFYPREAKVQWKVDNALQSGNSQESVTEQDSKDSTYSLSSTLTLSKADYEKHKVYACEVTHQGLSSPVTKSFNRGEC